European Patent Application EP 4 209 596 A1, published July 12, 2023. Title: ELECTROCHEMICAL SYSTEM FOR THE RAPID AND SENSITIVE DETECTION AND QUANTIFICATION OF NUCLEASE-LIKE ACTIVITY EXHIBITING ENZYMES. Applicant: UAB "Bioanalizes sistemos" UAB "Laboratorija 1". The sequence listing filed with the application follows.

SEQUENCE LISTING (4 sequences)

SEQ ID NO: 1 - DNA, 18 bp, Artificial Sequence
  Short chain
cgactactgctctcgggc

SEQ ID NO: 2 - DNA, 43 bp, Artificial Sequence
  Long chain
gcccgagagcagtagtcgttaagtctgtttgtgtttgataatt

SEQ ID NO: 3 - DNA, 25 bp, Artificial Sequence
  Probe
aattatcaaacacaaacagacttaa

SEQ ID NO: 4 - RNA, 43 nt, Artificial Sequence
  Target
ggcagggcagggcagucguuaagucuguuuguguuugauaauu